European Patent Specification EP 3 784 269 B1, published June 5, 2024. Title: Integrin Targeting Ligands and Uses Thereof. Applicant: ARROWHEAD PHARMACEUTICALS, INC. The sequence listing filed with the application follows.

SEQUENCE LISTING (6 sequences)

SEQ ID NO: 1 - RNA, 21 nt, Homo sapiens
  RNAi agent antisense strand modified sequence
uuucaugaaaucguuacguug

SEQ ID NO: 2 - RNA, 21 nt, Artificial sequence
  RNAi agent sense strand modified sequence
caacguaacgauuucaugaaa

SEQ ID NO: 3 - RNA, 21 nt, Artificial sequence
  RNAi agent antisense strand modified sequence
uuucaugaaaucguuacguug

SEQ ID NO: 4 - RNA, 21 nt, Artificial sequence
  RNAi agent sense strand modified sequence
caacguaacgauuucaugaaa

SEQ ID NO: 5 - RNA, 21 nt, Artificial sequence
  RNAi agent antisense strand modified sequence
uuucaugaaaucguuacguug

SEQ ID NO: 6 - RNA, 21 nt, Artificial sequence
  RNAi agent sense strand modified sequence
caacguaacgauuucaugaaa